European Patent Application EP 4 755 899 A1, published June 10, 2026. Title: An immunoanalytical method using Treponema pallidum antigen 47kDa (TpN47) as an antigen. Applicant: Denka Co. Ltd. The sequence listing filed with the application follows.

SEQUENCE LISTING (5 sequences)

SEQ ID NO: 1 - protein, 434 aa, Treponema pallidum
MKVKYALLSAGALQLLVVGCGSSHHETHYGYATLSYADYWAGELGQSRDVLLAGNAEADRAGDLDAGMFDAVSRATHGHGAFRQQFQYAVEVLGEKVLSKQETEDSRGRKKWEYETDPSVTKMVRASASFQDLGEDGEIKFEAVEGAVALADRASSFMVDSEEYKITNVKVHGMKFVPVAVPHELKGIAKEKFHFVEDSRVTENTNGLKTMLTEDSFSARKVSSMESPHDLVVDTVGTGYHSRFGSDAEASVMLKRADGSELSHREFIDYVMNFNTVRYDYYGDDASYTNLMASYGTKHSADSWWKTGRVPRISCGINYGFDRFKGSGPGYYRLTLIANGYRDVVADVRFLPKYEGNIDIGLKGKVLTIGGADAETLMDAAVDVFADGQPKLVSDQAVSLGQNVLSADFTPGTEYTVEVRFKEFGSVRAKVVAQ

SEQ ID NO: 2 - protein, 414 aa, synthetic construct
  REGION 1..414: note = Synthetic
GSSHHETHYGYATLSYADYWAGELGQSRDVLLAGNAEADRAGDLDAGMFDAVSRATHGHGAFRQQFQYAVEVLGEKVLSKQETEDSRGRKKWEYETDPSVTKMVRASASFQDLGEDGEIKFEAVEGAVALADRASSFMVDSEEYKITNVKVHGMKFVPVAVPHELKGIAKEKFHFVEDSRVTENTNGLKTMLTEDSFSARKVSSMESPHDLVVDTVGTGYHSRFGSDAEASVMLKRADGSELSHREFIDYVMNFNTVRYDYYGDDASYTNLMASYGTKHSADSWWKTGRVPRISCGINYGFDRFKGSGPGYYRLTLIANGYRDVVADVRFLPKYEGNIDIGLKGKVLTIGGADAETLMDAAVDVFADGQPKLVSDQAVSLGQNVLSADFTPGTEYTVEVRFKEFGSVRAKVVAQ

SEQ ID NO: 3 - protein, 331 aa, synthetic construct
  REGION 1..331: note = Synthetic
GSSHHETHYGYATLSYADYWAGELGQSRDVLLAGNAEADRAGDLDAGMFDAVSRATHGHGAFRQQFQYAVEVLGEKVLSKQETEDSRGRKKWEYETDPSVTKMVRASASFQDLGEDGEIKFEAVEGAVALADRASSFMVDSEEYKITNVKVHGMKFVPVAVPHELKGIAKEKFHFVEDSRVTENTNGLKTMLTEDSFSARKVSSMESPHDLVVDTVGTGYHSRFGSDAEASVMLKRADGSELSHREFIDYVMNFNTVRYDYYGDDASYTNLMASYGTKHSADSWWKTGRVPRISCGINYGFDRFKGSGPGYYRLTLIANGYRDVVADVRFL

SEQ ID NO: 4 - protein, 294 aa, synthetic construct
  REGION 1..294: note = Synthetic
GSSHHETHYGYATLSYADYWAGELGQSRDVLLAGNAEADRAGDLDAGMFDAVSRATHGHGAFRQQFQYAVEVLGEKVLSKQETEDSRGRKKWEYETDPSVTKMVRASASFQDLGEDGEIKFEAVEGAVALADRASSFMVDSEEYKITNVKVHGMKFVPVAVPHELKGIAKEKFHFVEDSRVTENTNGLKTMLTEDSFSARKVSSMESPHDLPKYEGNIDIGLKGKVLTIGGADAETLMDAAVDVFADGQPKLVSDQAVSLGQNVLSADFTPGTEYTVEVRFKEFGSVRAKVVAQ

SEQ ID NO: 5 - protein, 83 aa, synthetic construct
  REGION 1..83: note = Synthetic
PKYEGNIDIGLKGKVLTIGGADAETLMDAAVDVFADGQPKLVSDQAVSLGQNVLSADFTPGTEYTVEVRFKEFGSVRAKVVAQ